European Patent Specification EP 3 584 576 B1, published May 22, 2024. Title: A method of identifying a target protein for drug discovery to contribute development of antibody drugs. Applicant: Mitsui Chemicals, inc.; National Institutes of Biomedical Innovation, Health and Nutrition; and Savid Therapeutics Inc. The sequence listing filed with the application follows.

SEQUENCE LISTING (36 sequences)

SEQ ID NO: 1 - protein, 159 aa, Streptomyces avidinii
  An amino acid sequence of a wild type streptavidin
DPSKDSKAQVSAAEAGITGTWYNQLGSTFIVTAGADGALTGTYESAVGNAESRYVLTGRYDSAPATDGSGTALGWTVAWKNNYRNAHSATTWSGQYVGGAEARINTQWLLTSGTTEANAWKSTLVGHDTFTKVKPSAASIDAAKKAGVNNGNPLDAVQQ

SEQ ID NO: 2 - protein, 127 aa, Streptomyces avidinii
  Truncated amino acid sequence of a wild type streptavidin
AEAGITGTWYNQLGSTFIVTAGADGALTGTYESAVGNAESRYVLTGRYDSAPATDGSGTALGWTVAWKNNYRNAHSATTWSGQYVGGAEARINTQWLLTSGTTEANAWKSTLVGHDTFTKVKPSAAS

SEQ ID NO: 3 - DNA, 44 bp, Artificial
  Forward primer for mutation
ttaccggcacctggtatgatcagctgggcagcacctttattgtg

SEQ ID NO: 4 - DNA, 44 bp, Artificial
  Reverse primer for mutation
aaggtgctgcccagctgatcataccaggtgccggtaatacctgc

SEQ ID NO: 5 - DNA, 45 bp, Artificial
  Forward primer for mutation
ggtatgatcagctgggcgcgacctttattgtgaccgccggcgcag

SEQ ID NO: 6 - DNA, 45 bp, Artificial
  Reverse primer for mutation
gcggtcacaataaaggtcgcgcccagctgatcataccaggtgccg

SEQ ID NO: 7 - DNA, 43 bp, Artificial
  Forward primer for mutation
tgaccggcacctatgaagcggccgtgggtaatgcggaaagccg

SEQ ID NO: 8 - DNA, 44 bp, Artificial
  Reverse primer for mutation
tccgcattacccacggccgcttcataggtgccggtcagcgcacc

SEQ ID NO: 9 - DNA, 43 bp, Artificial
  Forward primer for mutation
tgaccggcacctatgaaaacgccgtgggtaatgcggaaagccg

SEQ ID NO: 10 - DNA, 44 bp, Artificial
  Reverse primer for mutation
tccgcattacccacggcgttttcataggtgccggtcagcgcacc

SEQ ID NO: 11 - DNA, 45 bp, Artificial
  Forward primer for mutation
atgaagcggccgtgggtggcgcggaaagccgttatgttctgaccg

SEQ ID NO: 12 - DNA, 45 bp, Artificial
  Reverse primer for mutation
acataacggctttccgcgccacccacggccgcttcataggtgccg

SEQ ID NO: 13 - DNA, 43 bp, Artificial
  Forward primer for mutation
caattatcgtaacgcccatggcgcgaccacctggagcggccag

SEQ ID NO: 14 - DNA, 43 bp, Artificial
  Reverse primer for mutation
gctccaggtggtcgcgccatgggcgttacgataattgtttttc

SEQ ID NO: 15 - DNA, 43 bp, Artificial
  Forward primer for mutation
caattatcgtaacgcccatcgtgcgaccacctggagcggccag

SEQ ID NO: 16 - DNA, 43 bp, Artificial
  Reverse primer for mutation
gctccaggtggtcgcacgatgggcgttacgataattgtttttc

SEQ ID NO: 17 - DNA, 43 bp, Artificial
  Forward primer for mutation
cccagtggctgctgaccctgggcaccaccgaagccaatgcgtg

SEQ ID NO: 18 - DNA, 43 bp, Artificial
  Reverse primer for mutation
ggcttcggtggtgcccagggtcagcagccactgggtgttaatg

SEQ ID NO: 19 - DNA, 43 bp, Artificial
  Forward primer for mutation
cccagtggctgctgaccattggcaccaccaatgccaatgcgtg

SEQ ID NO: 20 - DNA, 43 bp, Artificial
  Reverse primer for mutation
ggcattggtggtgccaatggtcagcagccactgggtgttaatg

SEQ ID NO: 21 - DNA, 43 bp, Artificial
  Forward primer for mutation
cccagtggctgctgaccgtgggcaccaccaatgccaatgcgtg

SEQ ID NO: 22 - DNA, 43 bp, Artificial
  Reverse primer for mutation
ggcattggtggtgcccacggtcagcagccactgggtgttaatg

SEQ ID NO: 23 - DNA, 43 bp, Artificial
  Forward primer for mutation
cccagtggctgctgaccatgggcaccaccaatgccaatgcgtg

SEQ ID NO: 24 - DNA, 44 bp, Artificial
  Reverse primer for mutation
ggcattcggtggtgcccatggtcagcagccactgggtgttaatg

SEQ ID NO: 25 - DNA, 43 bp, Artificial
  Forward primer for mutation
cccagtggctgctgacccgtggcaccaccgaagccaatgcgtg

SEQ ID NO: 26 - DNA, 43 bp, Artificial
  Reverse primer for mutation
ggcttcggtggtgccacgggtcagcagccactgggtgttaatg

SEQ ID NO: 27 - DNA, 43 bp, Artificial
  Forward primer for mutation
ccgaagccaatgcgtggatgagcaccctggtgggtcatgatac

SEQ ID NO: 28 - DNA, 43 bp, Artificial
  Reverse primer for mutation
tgacccaccagggtgctcatccacgcattggcttcggtggtgc

SEQ ID NO: 29 - DNA, 43 bp, Artificial
  Forward primer for mutation
ccgaagccaatgcgtggcgtagcaccctggtgggtcatgatac

SEQ ID NO: 30 - DNA, 43 bp, Artificial
  Reverse primer for mutation
tgacccaccagggtgctacgccacgcattggcttcggtggtgc

SEQ ID NO: 31 - DNA, 43 bp, Artificial
  Forward primer for mutation
ccgaagccaatgcgtgggaaagcaccctggtgggtcatgatac

SEQ ID NO: 32 - DNA, 43 bp, Artificial
  Reverse primer for mutation
tgacccaccagggtgctttcccacgcattggcttcggtggtgc

SEQ ID NO: 33 - DNA, 43 bp, Artificial
  Forward primer for mutation
caatgcgtggaaaagcaccaacgtgggtcatgatacctttacc

SEQ ID NO: 34 - DNA, 43 bp, Artificial
  Reverse primer for mutation
aggtatcatgacccacgttggtgcttttccacgcattggcttc

SEQ ID NO: 35 - DNA, 43 bp, Artificial
  Forward primer for mutation
caatgcgtggaaaagcacccaggtgggtcatgatacctttacc

SEQ ID NO: 36 - DNA, 43 bp, Artificial
  Reverse primer for mutation
aggtatcatgacccacctgggtgcttttccacgcattggcttc